European Patent Application EP 4 574 957 A1, published June 25, 2025. Title: Dispersin- und Cellulase-haltiges Waschmittel mit verbesserter Lagerstabilität. Applicant: Henkel AG & Co. KGaA. The sequence listing filed with the application follows.

SEQUENCE LISTING (1 sequence)

SEQ ID NO: 1 - protein, 324 aa, Terribacillus saccharophilus [sequence omitted]